European Patent Specification EP 3 731 875 B1, published October 4, 2023. Title: MONOSPECIFIC AND BISPECIFIC PROTEINS WITH IMMUNE CHECKPOINT REGULATION FOR CANCER THERAPY. Applicant: HER, JENG-HORNG. The sequence listing filed with the application follows.

SEQUENCE LISTING (43 sequences)

SEQ ID NO: 1 - protein, 217 aa, Homo sapiens
QSVLTQPPSASGTPGQRVTISCSGSSSNIGSNTVNWYQQLPGTAPKLLIYSNNQRPSGVPDRFSGSKSGTSASLAISGLQSEDEADYYCATWDDSLNAWVVFGGGTKLTVLGQPKAAPSVTLFPPSSEELQANKATLVCLISDFYPGAVTVAWKADSSPVKAGVETTTPSKQSNNKYAASSYLSLTPEQWKSHRSYSCQVTHEGSTVEKTVAPTECS

SEQ ID NO: 2 - protein, 118 aa, Homo sapiens
QVQLVQSGAEVKKPGSSVKVSCKASGGTFRRYSISWVRQAPGQGLEWMGGIIPVFGAAKYAQKFQGRVTITADEFTSTAYMELSSLTSEDTAVYYCALSGDSDAFDIWGQGTMVTVSS

SEQ ID NO: 3 - protein, 216 aa, Homo sapiens
QSALTQPASVSGSPGQSITISCTGTSNDVGSYNSVSWYQQHPGKAPKLVIYEVANRPSGVPDRFSGSKSGNTASLTISGLQAEDEADYYCSSYTSSSTLVFGGGTKLTVLGQPKAAPSVTLFPPSSEELQANKATLVCLISDFYPGAVTVAWKADSSPVKAGVETTTPSKQSNNKYAASSYLSLTPEQWKSHRSYSCQVTHEGSTVEKTVAPTECS

SEQ ID NO: 4 - protein, 121 aa, Homo sapiens
QVQLVQSGAKVKKPGSSVKVSCKASGGTFSSYAISWVRQAPGQGLEWMGRIIPILGIANYAQKFQGRVTITADKSTSTAYMELSSLRSEDTAVYYCARVVPGYSYGPFDYWGQGTTVTVSS

SEQ ID NO: 5 - protein, 214 aa, Homo sapiens
SYVLTQPPSVSVTPGKTARIACGGNNLESKIVSWYQQKPGQAPVLVIFYDTDRPSGISERFSGSNSGNTATLTISRVEAGDEADYYCQVWDSNSDHVIFGGGTKLTVLGQPKAAPSVTLFPPSSEELQANKATLVCLISDFYPGAVTVAWKADSSPVKAGVETTTPSKQSNNKYAASSYLSLTPEQWKSHRSYSCQVTHEGSTVEKTVAPTECS

SEQ ID NO: 6 - protein, 126 aa, Homo sapiens
EVQLVESGGVVVQPGGSLRLSCAASGFTFDDYTMHWVRQAPGKGLEWVSLISWDGGSTYYADSVKGRFTISRDNSKNSLYLQMNSLRTEDTALYYCASIYDPPPGSRSALDAFDIWGQGTMVTVSS

SEQ ID NO: 7 - protein, 214 aa, Homo sapiens
SYVLTQPPSVSVTPGKTARIACGGNNLESKIVSWYQQKPGQAPVLVIFYDTDRPSGISERFSGSNSGNTATLTISRVEAGDEADYYCQVWDSNSDHVIFGGGTKLTVLGQPKAAPSVTLFPPSSEELQANKATLVCLISDFYPGAVTVAWKADSSPVKAGVETTTPSKQSNNKYAASSYLSLTPEQWKSHRSYSCQVTHEGSTVEKTVAPAECS

SEQ ID NO: 8 - protein, 118 aa, Homo sapiens
EVQLVESGGGLVKPGGSLRLSCAASGFTFSSYSMNWVRQAPGKGLEWVSSISSSSRYIYYADSVKGRFTISRDNAKNSLYLQMNSLRAEDTAVYYCARQNEDVAFGIWGQGTMVTVSS

SEQ ID NO: 9 - protein, 327 aa, Homo sapiens
ASTKGPSVFPLAPCSRSTSESTAALGCLVKDYFPEPVTVSWNSGALTSGVHTFPAVLQSSGLYSLSSVVTVPSSSLGTKTYTCNVDHKPSNTKVDKRVESKYGPPCPPCPAPEFLGGPSVFLFPPKPKDTLMISRTPEVTCVVVDVSQEDPEVQFNWYVDGVEVHNAKTKPREEQFNSTYRVVSVLTVLHQDWLNGKEYKCKVSNKGLPSSIEKTISKAKGQPREPQVYTLPPSQEEMTKNQVSLTCLVKGFYPSDIAVEWESNGQPENNYKTTPPVLDSDGSFFLYSRLTVDKSRWQEGNVFSCSVMHEALHNHYTQKSLSLSLGK

SEQ ID NO: 10 - protein, 246 aa, Artificial Sequence
  OX40 scFv (Clone A4)
QSALTQPPSASGSPGQSVTISCTGTSSDVGGYNYVSWYQQHPGKAPKLMIYEVSQRPSGVPDRFSGSKSGNTASLTVSGLQAEDEADYYCSSYAGSNNLGVFGGGTKLTVSSGGGGSGGGGSGGGGSQVQLVESGGGLVQPGGSLRLSCAASGFTFSSYEMNWVRQAPGKGLEWVSYISSSGSTIYYADSVKGRFTISRDNAKNSLYLQMNSLRAEDTAVYYCARGGVGDAFDIWGQGTMVTVSSA

SEQ ID NO: 11 - protein, 250 aa, Artificial Sequence
  OX40 scFv (Clone B17)
YVLTQPPSVSVTPGKTARIACGGNNLESKIVSWYQQKPGQAPVLVIFYDTDRPSGISERFSGSNSGNTATLTISRVEAGDEADYYCQVWDSNSDHVIFGGGTKLTVSSGGGGSGGGGSGGGGSEVQLVESGGVVVQPGGSLRLSCAASGFTFDDYTMHWVRQAPGKGLEWVSLISWDGGSTYYADSVKGRFTISRDNSKNSLYLQMNSLRTEDTALYYCASIYDPPPGSRSALDAFDIWGQGTMVTVSSA

SEQ ID NO: 12 - protein, 243 aa, Artificial Sequence
  OX40 scFv (Clone B19)
SYVLTQPPSVSVTPGKTARIACGGNNLESKIVSWYQQKPGQAPVLVIFYDTDRPSGISERFSGSNSGNTATLTISRVEAGDEADYYCQVWDSNSDHVIFGGGTKLTVSSGGGGSGGGGSGGGGSEVQLVESGGGLVKPGGSLRLSCAASGFTFSSYSMNWVRQAPGKGLEWVSSISSSSRYIYYADSVKGRFTISRDNAKNSLYLQMNSLRAEDTAVYYCARQNEDVAFGIWGQGTMVTVSSA

SEQ ID NO: 13 - protein, 241 aa, Artificial Sequence
  OX40 scFv (Clone B120)
SYELTQPPSVSVSPGQTASITCSGDTLGDKYASWYQQKPGRSPVLVIYQDSERPSGIPERFSGSNSGNTATLTISGTQAMDEADYYCQAWDSSTSYVFGTGTKVTVSSGGGGSGGGGSGGGGSQVQLQQWGAGLLKPSETLSLTCAVYGGSFSGYYWSWIRQPPGKGLEWIGEINHSGSTNYNPSLKSRVTISVDTSKNQFSLKLSSVTAADTAVYYCARGRWGGSFIYWGQGTLVTVSSA

SEQ ID NO: 14 - protein, 6 aa, Artificial Sequence
  peptide linker
GGGGGS

SEQ ID NO: 15 - protein, 20 aa, Artificial Sequence
  signal peptide
METDTLLLWVLLLWVPGSTG

SEQ ID NO: 16 - protein, 704 aa, Artificial Sequence
  Anti-PD-L1-clone 6 Heavy Chain-OX40 clone B17 scFv antibody
QVQLVQSGAEVKKPGSSVKVSCKASGGTFRRYSISWVRQAPGQGLEWMGGIIPVFGAAKYAQKFQGRVTITADEFTSTAYMELSSLTSEDTAVYYCALSGDSDAFDIWGQGTMVTVSSASTKGPSVFPLAPCSRSTSESTAALGCLVKDYFPEPVTVSWNSGALTSGVHTFPAVLQSSGLYSLSSVVTVPSSSLGTKTYTCNVDHKPSNTKVDKRVESKYGPPCPPCPAPEFLGGPSVFLFPPKPKDTLMISRTPEVTCVVVDVSQEDPEVQFNWYVDGVEVHNAKTKPREEQFNSTYRVVSVLTVLHQDWLNGKEYKCKVSNKGLPSSIEKTISKAKGQPREPQVYTLPPSQEEMTKNQVSLTCLVKGFYPSDIAVEWESNGQPENNYKTTPPVLDSDGSFFLYSRLTVDKSRWQEGNVFSCSVMHEALHNHYTQKSLSLSLGGGGGSGGGGSYVLTQPPSVSVTPGKTARIACGGNNLESKIVSWYQQKPGQAPVLVIFYDTDRPSGISERFSGSNSGNTATLTISRVEAGDEADYYCQVWDSNSDHVIFGGGTKLTVSSGGGGSGGGGSGGGGSEVQLVESGGVVVQPGGSLRLSCAASGFTFDDYTMHWVRQAPGKGLEWVSLISWDGGSTYYADSVKGRFTISRDNSKNSLYLQMNSLRTEDTALYYCASIYDPPPGSRSALDAFDIWGQGTMVTVSSA

SEQ ID NO: 17 - protein, 696 aa, Artificial Sequence
  Anti-PD-L1-clone  6 Heavy Chain-OX40 clone B19 scFv antibody
QVQLVQSGAEVKKPGSSVKVSCKASGGTFRRYSISWVRQAPGQGLEWMGGIIPVFGAAKYAQKFQGRVTITADEFTSTAYMELSSLTSEDTAVYYCALSGDSDAFDIWGQGTMVTVSSASTKGPSVFPLAPCSRSTSESTAALGCLVKDYFPEPVTVSWNSGALTSGVHTFPAVLQSSGLYSLSSVVTVPSSSLGTKTYTCNVDHKPSNTKVDKRVESKYGPPCPPCPAPEFLGGPSVFLFPPKPKDTLMISRTPEVTCVVVDVSQEDPEVQFNWYVDGVEVHNAKTKPREEQFNSTYRVVSVLTVLHQDWLNGKEYKCKVSNKGLPSSIEKTISKAKGQPREPQVYTLPPSQEEMTKNQVSLTCLVKGFYPSDIAVEWESNGQPENNYKTTPPVLDSDGSFFLYSRLTVDKSRWQEGNVFSCSVMHEALHNHYTQKSLSLSLGGGGGSGGGGSYVLTQPPSVSVTPGKTARIACGGNNLESKIVSWYQQKPGQAPVLVIFYDTDRPSGISERFSGSNSGNTATLTISRVEAGDEADYYCQVWDSNSDHVIFGGGTKLTVSSGGGGSGGGGSGGGGSEVQLVESGGGLVKPGGSLRLSCAASGFTFSSYSMNWVRQAPGKGLEWVSSISSSSRYIYYADSVKGRFTISRDNAKNSLYLQMNSLRAEDTAVYYCARQNEDVAFGIWGQGTMVTVSSA

SEQ ID NO: 18 - protein, 707 aa, Artificial Sequence
  Anti-PD-L1-OX40 Ab-V1
QVQLVQSGAEVKKPGSSVKVSCKASGGTFRRYSISWVRQAPGQGLEWMGGIIPVFGAAKYAQKFQGRVTITADEFTSTAYMELSSLTSEDTAVYYCALSGDSDAFDIWGQGTMVTVSSASTKGPSVFPLAPCSRSTSESTAALGCLVKDYFPEPVTVSWNSGALTSGVHTFPAVLQSSGLYSLSSVVTVPSSSLGTKTYTCNVDHKPSNTKVDKRVESKYGPPCPPCPAPEFLGGPSVFLFPPKPKDTLMISRTPEVTCVVVDVSQEDPEVQFNWYVDGVEVHNAKTKPREEQFNSTYRVVSVLTVLHQDWLNGKEYKCKVSNKGLPSSIEKTISKAKGQPREPQVYTLPPSQEEMTKNQVSLTCLVKGFYPSDIAVEWESNGQPENNYKTTPPVLDSDGSFFLYSRLTVDKSRWQEGNVFSCSVMHEALHNHYTQKSLSLSLGGGGGSGGGGSYVLTQPPSVSVTPGKTARIACGGNNLESKIVSWYQQKPGQAPVLVIFYDTDRPSGISERFSGSNSGNTATLTISRVEAGDEADYYCQVWDSNSDHVIFGGGTKLTVLSSGGGGSGGGGGGSSRSSLEVQLVESGGVVVQPGGSLRLSCAASGFTFDDYTMHWVRQAPGKGLEWVSLISWDGGSTYYADSVKGRFTISRDNSKNSLYLQMNSLRTEDTALYYCASIYDPPPGSRSALDAFDIWGQGTMVTVSSA

SEQ ID NO: 19 - protein, 708 aa, Artificial Sequence
  Anti-PD-L1-OX40 Ab-V2
QVQLVQSGAEVKKPGSSVKVSCKASGGTFRRYSISWVRQAPGQGLEWMGGIIPVFGAAKYAQKFQGRVTITADEFTSTAYMELSSLTSEDTAVYYCALSGDSDAFDIWGQGTMVTVSSASTKGPSVFPLAPCSRSTSESTAALGCLVKDYFPEPVTVSWNSGALTSGVHTFPAVLQSSGLYSLSSVVTVPSSSLGTKTYTCNVDHKPSNTKVDKRVESKYGPPCPPCPAPEFLGGPSVFLFPPKPKDTLMISRTPEVTCVVVDVSQEDPEVQFNWYVDGVEVHNAKTKPREEQFNSTYRVVSVLTVLHQDWLNGKEYKCKVSNKGLPSSIEKTISKAKGQPREPQVYTLPPSQEEMTKNQVSLTCLVKGFYPSDIAVEWESNGQPENNYKTTPPVLDSDGSFFLYSRLTVDKSRWQEGNVFSCSVMHEALHNHYTQKSLSLSLGGGGGSGGGGSYVLTQPPSVSVTPGKTARIACGGNNLESKIVSWYQQKPGQAPVLVIFYDTDRPSGISERFSGSNSGNTATLTISRVEAGDEADYYCQVWDSNSDHVIFGGGTKLTVLGGKGSGGKGTGGKGSGGKGSEVQLVESGGVVVQPGGSLRLSCAASGFTFDDYTMHWVRQAPGKGLEWVSLISWDGGSTYYADSVKGRFTISRDNSKNSLYLQMNSLRTEDTALYYCASIYDPPPGSRSALDAFDIWGQGTMVTVSSA

SEQ ID NO: 20 - protein, 701 aa, Artificial Sequence
  Anti-PD-L1-OX40 Ab-V3
QVQLVQSGAEVKKPGSSVKVSCKASGGTFRRYSISWVRQAPGQGLEWMGGIIPVFGAAKYAQKFQGRVTITADEFTSTAYMELSSLTSEDTAVYYCALSGDSDAFDIWGQGTMVTVSSASTKGPSVFPLAPCSRSTSESTAALGCLVKDYFPEPVTVSWNSGALTSGVHTFPAVLQSSGLYSLSSVVTVPSSSLGTKTYTCNVDHKPSNTKVDKRVESKYGPPCPPCPAPEFLGGPSVFLFPPKPKDTLMISRTPEVTCVVVDVSQEDPEVQFNWYVDGVEVHNAKTKPREEQFNSTYRVVSVLTVLHQDWLNGKEYKCKVSNKGLPSSIEKTISKAKGQPREPQVYTLPPSQEEMTKNQVSLTCLVKGFYPSDIAVEWESNGQPENNYKTTPPVLDSDGSFFLYSRLTVDKSRWQEGNVFSCSVMHEALHNHYTQKSLSLSLGGGGGSGGGGSYVLTQPPSVSVTPGKTARIACGGNNLESKIVSWYQQKPGQAPVLVIFYDTDRPSGISERFSGSNSGNTATLTISRVEAGDEADYYCQVWDSNSDHVIFGGGTKLTVLGSASAPTLFPLVSEVQLVESGGVVVQPGGSLRLSCAASGFTFDDYTMHWVRQAPGKGLEWVSLISWDGGSTYYADSVKGRFTISRDNSKNSLYLQMNSLRTEDTALYYCASIYDPPPGSRSALDAFDIWGQGTMVTVSSA

SEQ ID NO: 21 - protein, 706 aa, Artificial Sequence
  Anti-PD-L1-OX40 Ab-V4
QVQLVQSGAEVKKPGSSVKVSCKASGGTFRRYSISWVRQAPGQGLEWMGGIIPVFGAAKYAQKFQGRVTITADEFTSTAYMELSSLTSEDTAVYYCALSGDSDAFDIWGQGTMVTVSSASTKGPSVFPLAPCSRSTSESTAALGCLVKDYFPEPVTVSWNSGALTSGVHTFPAVLQSSGLYSLSSVVTVPSSSLGTKTYTCNVDHKPSNTKVDKRVESKYGPPCPPCPAPEFLGGPSVFLFPPKPKDTLMISRTPEVTCVVVDVSQEDPEVQFNWYVDGVEVHNAKTKPREEQFNSTYRVVSVLTVLHQDWLNGKEYKCKVSNKGLPSSIEKTISKAKGQPREPQVYTLPPSQEEMTKNQVSLTCLVKGFYPSDIAVEWESNGQPENNYKTTPPVLDSDGSFFLYSRLTVDKSRWQEGNVFSCSVMHEALHNHYTQKSLSLSLGGGGGSGGGGSYVLTQPPSVSVTPGKTARIACGGNNLESKIVSWYQQKPGQAPVLVIFYDTDRPSGISERFSGSNSGNTATLTISRVEAGDEADYYCQVWDSNSDHVIFGGGTKLTVLGSTSGSGKPGSGEGSTKGEVQLVESGGVVVQPGGSLRLSCAASGFTFDDYTMHWVRQAPGKGLEWVSLISWDGGSTYYADSVKGRFTISRDNSKNSLYLQMNSLRTEDTALYYCASIYDPPPGSRSALDAFDIWGQGTMVTVSSA

SEQ ID NO: 22 - protein, 706 aa, Artificial Sequence
  Anti-PD-L1-OX40 Ab-V5
QVQLVQSGAEVKKPGSSVKVSCKASGGTFRRYSISWVRQAPGQGLEWMGGIIPVFGAAKYAQKFQGRVTITADEFTSTAYMELSSLTSEDTAVYYCALSGDSDAFDIWGQGTMVTVSSASTKGPSVFPLAPCSRSTSESTAALGCLVKDYFPEPVTVSWNSGALTSGVHTFPAVLQSSGLYSLSSVVTVPSSSLGTKTYTCNVDHKPSNTKVDKRVESKYGPPCPPCPAPEFLGGPSVFLFPPKPKDTLMISRTPEVTCVVVDVSQEDPEVQFNWYVDGVEVHNAKTKPREEQFNSTYRVVSVLTVLHQDWLNGKEYKCKVSNKGLPSSIEKTISKAKGQPREPQVYTLPPSQEEMTKNQVSLTCLVKGFYPSDIAVEWESNGQPENNYKTTPPVLDSDGSFFLYSRLTVDKSRWQEGNVFSCSVMHEALHNHYTQKSLSLSLGGGGGSGGGGSYELTQPPSVSVTPGQTARIACGGNNLESKIVSWYQQKPGQAPVLVIFYDTDRPSGISERFSGSNSGNTATLTISRVEAGDEADYYCQVWDSNSDHVIFGGGTKLTVLGSTSGSGKPGSGEGSTKGEVQLVESGGVVVQPGGSLRLSCAASGFTFDDYTMHWVRQAPGKGLEWVSLISWDGGSTYYADSVKGRFTISRDNSKNSLYLQMNSLRTEDTALYYCASIYDPPPGSRSALDAFDIWGQGTMVTVSSA

SEQ ID NO: 23 - protein, 706 aa, Artificial Sequence
  Anti-PD-L1-OX40 Ab-V6
QVQLVQSGAEVKKPGSSVKVSCKASGGTFRRYSISWVRQAPGQGLEWMGGIIPVFGAAKYAQKFQGRVTITADEFTSTAYMELSSLTSEDTAVYYCALSGDSDAFDIWGQGTMVTVSSASTKGPSVFPLAPCSRSTSESTAALGCLVKDYFPEPVTVSWNSGALTSGVHTFPAVLQSSGLYSLSSVVTVPSSSLGTKTYTCNVDHKPSNTKVDKRVESKYGPPCPPCPAPEFLGGPSVFLFPPKPKDTLMISRTPEVTCVVVDVSQEDPEVQFNWYVDGVEVHNAKTKPREEQFNSTYRVVSVLTVLHQDWLNGKEYKCKVSNKGLPSSIEKTISKAKGQPREPQVYTLPPSQEEMTKNQVSLTCLVKGFYPSDIAVEWESNGQPENNYKTTPPVLDSDGSFFLYSRLTVDKSRWQEGNVFSCSVMHEALHNHYTQKSLSLSLGGGGGSGGGGSYVLTQPPSVSVTPGETARIACGGNNLESKIVSWYQQKPGQAPVLVIFYDTDRPSGISERFSGSNSGNTATLTISRVEAGDEADYYCQVWDSNSDHVVFGGGTKLTVLGSTSGSGKPGSGEGSTKGEVQLVESGGGVVQPGGSLRLSCAASGFTFDDYTMHWVRQAPGKGLEWVSLISWDGGSTYYADSVKGRFTISRDNSKNSLYLQMNSLRTEDTALYYCASIYDPPPGSRSALDAFDIWGQGTMVTVSSA

SEQ ID NO: 24 - protein, 706 aa, Artificial Sequence
  Anti-PD-L1-OX40 Ab-V7
QVQLVQSGAEVKKPGSSVKVSCKASGGTFRRYSISWVRQAPGQGLEWMGGIIPVFGAAKYAQKFQGRVTITADEFTSTAYMELSSLTSEDTAVYYCALSGDSDAFDIWGQGTMVTVSSASTKGPSVFPLAPCSRSTSESTAALGCLVKDYFPEPVTVSWNSGALTSGVHTFPAVLQSSGLYSLSSVVTVPSSSLGTKTYTCNVDHKPSNTKVDKRVESKYGPPCPPCPAPEFLGGPSVFLFPPKPKDTLMISRTPEVTCVVVDVSQEDPEVQFNWYVDGVEVHNAKTKPREEQFNSTYRVVSVLTVLHQDWLNGKEYKCKVSNKGLPSSIEKTISKAKGQPREPQVYTLPPSQEEMTKNQVSLTCLVKGFYPSDIAVEWESNGQPENNYKTTPPVLDSDGSFFLYSRLTVDKSRWQEGNVFSCSVMHEALHNHYTQKSLSLSLGGGGGSGGGGSYVLTQPPSVSVTPGQTARIACGGNNLESKIVSWYQQKPGQAPVLVIFYDTDRPSGISERFSGSNSGNTATLTISRVEAGDEADYYCQVWDSNSDHVVFGGGTKLTVLGSTSGSGKPGSGEGSTKGEVQLVESGGGVVQPGGSLRLSCAASGFTFDDYTMHWVRQAPGKGLEWVSLISWDGGSTYYADSVKGRFTISRDNSKNSLYLQMNSLRTEDTALYYCASIYDPPPGSRSALDAFDIWGQGTMVTVSSA

SEQ ID NO: 25 - protein, 706 aa, Artificial Sequence
  Anti-PD-L1-OX40 Ab-V8
QVQLVQSGAEVKKPGSSVKVSCKASGGTFRRYSISWVRQAPGQGLEWMGGIIPVFGAAKYAQKFQGRVTITADEFTSTAYMELSSLTSEDTAVYYCALSGDSDAFDIWGQGTMVTVSSASTKGPSVFPLAPCSRSTSESTAALGCLVKDYFPEPVTVSWNSGALTSGVHTFPAVLQSSGLYSLSSVVTVPSSSLGTKTYTCNVDHKPSNTKVDKRVESKYGPPCPPCPAPEFLGGPSVFLFPPKPKDTLMISRTPEVTCVVVDVSQEDPEVQFNWYVDGVEVHNAKTKPREEQFNSTYRVVSVLTVLHQDWLNGKEYKCKVSNKGLPSSIEKTISKAKGQPREPQVYTLPPSQEEMTKNQVSLTCLVKGFYPSDIAVEWESNGQPENNYKTTPPVLDSDGSFFLYSRLTVDKSRWQEGNVFSCSVMHEALHNHYTQKSLSLSLGGGGGSGGGGSYVLTQPPSVSVAPGKTARITCGGNNLESKIVSWYQQKPGQAPVLVIFYDTDRPSGIPERFSGSNSGNTATLTISRVEAGDEADYYCQVWDSNSDHVIFGGGTKLTVLGSTSGSGKPGSGEGSTKGEVQLVESGGIVVQPGGSLRLSCAASGFTFDDYTMHWVRQAPGKGLEWVSLISWDGGSTYYADSVKGRFTISRDNSKNSLYLQMNSLRTEDTALYYCASIYDPPPGSRSALDAFDIWGQGTMVTVSSA

SEQ ID NO: 26 - protein, 706 aa, Artificial Sequence
  Anti-PD-L1-OX40 Ab-V9
QVQLVQSGAEVKKPGSSVKVSCKASGGTFRRYSISWVRQAPGQGLEWMGGIIPVFGAAKYAQKFQGRVTITADEFTSTAYMELSSLTSEDTAVYYCALSGDSDAFDIWGQGTMVTVSSASTKGPSVFPLAPCSRSTSESTAALGCLVKDYFPEPVTVSWNSGALTSGVHTFPAVLQSSGLYSLSSVVTVPSSSLGTKTYTCNVDHKPSNTKVDKRVESKYGPPCPPCPAPEFLGGPSVFLFPPKPKDTLMISRTPEVTCVVVDVSQEDPEVQFNWYVDGVEVHNAKTKPREEQFNSTYRVVSVLTVLHQDWLNGKEYKCKVSNKGLPSSIEKTISKAKGQPREPQVYTLPPSQEEMTKNQVSLTCLVKGFYPSDIAVEWESNGQPENNYKTTPPVLDSDGSFFLYSRLTVDKSRWQEGNVFSCSVMHEALHNHYTQKSLSLSLGGGGGSGGGGSYVLTQPPSVSVAPGKTARITCGGNNLESKIVSWYQQKPGQAPVLVIFYDTDRPSGIPERFSGSNSGNTATLTISRVEAGDEADYYCQVWDSNSDHVVFGGGTKLTVLGSTSGSGKPGSGEGSTKGEVQLVESGGGVVQPGGSLRLSCAASGFTFDDYTMHWVRQAPGKGLEWVSLISWDGGSTYYADSVKGRFTISRDNSKNSLYLQMNSLRTEDTALYYCASIYDPPPGSRSALDAFDIWGQGTMVTVSSA

SEQ ID NO: 27 - protein, 706 aa, Artificial Sequence
  Anti-PD-L1-OX40 Ab-V10
QVQLVQSGAEVKKPGSSVKVSCKASGGTFRRYSISWVRQAPGQGLEWMGGIIPVFGAAKYAQKFQGRVTITADEFTSTAYMELSSLTSEDTAVYYCALSGDSDAFDIWGQGTMVTVSSASTKGPSVFPLAPCSRSTSESTAALGCLVKDYFPEPVTVSWNSGALTSGVHTFPAVLQSSGLYSLSSVVTVPSSSLGTKTYTCNVDHKPSNTKVDKRVESKYGPPCPPCPAPEFLGGPSVFLFPPKPKDTLMISRTPEVTCVVVDVSQEDPEVQFNWYVDGVEVHNAKTKPREEQFNSTYRVVSVLTVLHQDWLNGKEYKCKVSNKGLPSSIEKTISKAKGQPREPQVYTLPPSQEEMTKNQVSLTCLVKGFYPSDIAVEWESNGQPENNYKTTPPVLDSDGSFFLYSRLTVDKSRWQEGNVFSCSVMHEALHNHYTQKSLSLSLGGGGGSGGGGSYVLTQPPSVSVAPGQTARITCGGNNLESKIVSWYQQKPGQAPVLVIFYDTDRPSGIPERFSGSNSGNTATLTISRVEAGDEADYYCQVWDSNSDHVVFGGGTKLTVLGSTSGSGKPGSGEGSTKGEVQLVESGGGVVQPGGSLRLSCAASGFTFDDYTMHWVRQAPGKGLEWVSLISWDGGSTYYADSVKGRFTISRDNSKNSLYLQMNSLRTEDTALYYCASIYDPPPGSRSALDAFDIWGQGTMVTVSSA

SEQ ID NO: 28 - protein, 706 aa, Artificial Sequence
  Anti-PD-L1-OX40 Ab-V11
QVQLVQSGAEVKKPGSSVKVSCKASGGTFRRYSISWVRQAPGQGLEWMGGIIPVFGAAKYAQKFQGRVTITADEFTSTAYMELSSLTSEDTAVYYCALSGDSDAFDIWGQGTMVTVSSASTKGPSVFPLAPCSRSTSESTAALGCLVKDYFPEPVTVSWNSGALTSGVHTFPAVLQSSGLYSLSSVVTVPSSSLGTKTYTCNVDHKPSNTKVDKRVESKYGPPCPPCPAPEFLGGPSVFLFPPKPKDTLMISRTPEVTCVVVDVSQEDPEVQFNWYVDGVEVHNAKTKPREEQFNSTYRVVSVLTVLHQDWLNGKEYKCKVSNKGLPSSIEKTISKAKGQPREPQVYTLPPSQEEMTKNQVSLTCLVKGFYPSDIAVEWESNGQPENNYKTTPPVLDSDGSFFLYSRLTVDKSRWQEGNVFSCSVMHEALHNHYTQKSLSLSLGGGGGSGGGGSYVLTQPPSVSVTPGETARIACGGNNLESKIVSWYQQKPGQAPVLVIFYDTDRPSGISERFSGSNSGNTATLTISRVEAGDEADYYCQVWDSNSDHVIFGGGTKLTVLGSTSGSGKPGSGEGSTKGEVQLVESGGVVVQPGGSLRLSCAASGFTFDDYTMHWVRQAPGKGLEWVSLISWDGGSTYYADSVKGRFTISRDNSKNSLYLQMNSLRTEDTALYYCASIYDPPPGSRSALDAFDIWGQGTMVTVSSA

SEQ ID NO: 29 - protein, 706 aa, Artificial Sequence
  Anti-PD-L1-OX40 Ab-V12
QVQLVQSGAEVKKPGSSVKVSCKASGGTFRRYSISWVRQAPGQGLEWMGGIIPVFGAAKYAQKFQGRVTITADEFTSTAYMELSSLTSEDTAVYYCALSGDSDAFDIWGQGTMVTVSSASTKGPSVFPLAPCSRSTSESTAALGCLVKDYFPEPVTVSWNSGALTSGVHTFPAVLQSSGLYSLSSVVTVPSSSLGTKTYTCNVDHKPSNTKVDKRVESKYGPPCPPCPAPEFLGGPSVFLFPPKPKDTLMISRTPEVTCVVVDVSQEDPEVQFNWYVDGVEVHNAKTKPREEQFNSTYRVVSVLTVLHQDWLNGKEYKCKVSNKGLPSSIEKTISKAKGQPREPQVYTLPPSQEEMTKNQVSLTCLVKGFYPSDIAVEWESNGQPENNYKTTPPVLDSDGSFFLYSRLTVDKSRWQEGNVFSCSVMHEALHNHYTQKSLSLSLGGGGGSGGGGSYVLTQPPSVSVTPGQTARIACGGNNLESKIVSWYQQKPGQAPVLVIFYDTDRPSGISERFSGSNSGNTATLTISRVEAGDEADYYCQVWDSNSDHVIFGGGTKLTVLGSTSGSGKPGSGEGSTKGEVQLVESGGVVVQPGGSLRLSCAASGFTFDDYTMHWVRQAPGKGLEWVSLISWDGGSTYYADSVKGRFTISRDNSKNSLYLQMNSLRTEDTALYYCASIYDPPPGSRSALDAFDIWGQGTMVTVSSA

SEQ ID NO: 30 - protein, 176 aa, Artificial Sequence
  Anti-PD-L1-OX40 Ab-V4
LSLGGGGGSGGGGSYVLTQPPSVSVTPGKTARIACGGNNLESKIVSWYQQKPGQAPVLVIFYDTDRPSGISERFSGSNSGNTATLTISRVEAGDEADYYCQVWDSNSDHVIFGGGTKLTVLGSTSGSGKPGSGEGSTKGEVQLVESGGVVVQPGGSLRLSCAASGFTFDDYTMHWV

SEQ ID NO: 31 - protein, 176 aa, Artificial Sequence
  Anti-PD-L1-OX40 Ab-V5
LSLGGGGGSGGGGSYELTQPPSVSVTPGQTARIACGGNNLESKIVSWYQQKPGQAPVLVIFYDTDRPSGISERFSGSNSGNTATLTISRVEAGDEADYYCQVWDSNSDHVIFGGGTKLTVLGSTSGSGKPGSGEGSTKGEVQLVESGGVVVQPGGSLRLSCAASGFTFDDYTMHWV

SEQ ID NO: 32 - protein, 176 aa, Artificial Sequence
  Anti-PD-L1-OX40 Ab-V6
LSLGGGGGSGGGGSYVLTQPPSVSVTPGETARIACGGNNLESKIVSWYQQKPGQAPVLVIFYDTDRPSGISERFSGSNSGNTATLTISRVEAGDEADYYCQVWDSNSDHVVFGGGTKLTVLGSTSGSGKPGSGEGSTKGEVQLVESGGGVVQPGGSLRLSCAASGFTFDDYTMHWV

SEQ ID NO: 33 - protein, 176 aa, Artificial Sequence
  Anti-PD-L1-OX40 Ab-V7
LSLGGGGGSGGGGSYVLTQPPSVSVTPGQTARIACGGNNLESKIVSWYQQKPGQAPVLVIFYDTDRPSGISERFSGSNSGNTATLTISRVEAGDEADYYCQVWDSNSDHVVFGGGTKLTVLGSTSGSGKPGSGEGSTKGEVQLVESGGGVVQPGGSLRLSCAASGFTFDDYTMHWV

SEQ ID NO: 34 - protein, 176 aa, Artificial Sequence
  Anti-PD-L1-OX40 Ab-V8
LSLGGGGGSGGGGSYVLTQPPSVSVAPGKTARITCGGNNLESKIVSWYQQKPGQAPVLVIFYDTDRPSGIPERFSGSNSGNTATLTISRVEAGDEADYYCQVWDSNSDHVIFGGGTKLTVLGSTSGSGKPGSGEGSTKGEVQLVESGGIVVQPGGSLRLSCAASGFTFDDYTMHWV

SEQ ID NO: 35 - protein, 176 aa, Artificial Sequence
  Anti-PD-L1-OX40 Ab-V9
LSLGGGGGSGGGGSYVLTQPPSVSVAPGKTARITCGGNNLESKIVSWYQQKPGQAPVLVIFYDTDRPSGIPERFSGSNSGNTATLTISRVEAGDEADYYCQVWDSNSDHVVFGGGTKLTVLGSTSGSGKPGSGEGSTKGEVQLVESGGGVVQPGGSLRLSCAASGFTFDDYTMHWV

SEQ ID NO: 36 - protein, 176 aa, Artificial Sequence
  Anti-PD-L1-OX40 Ab-V10
LSLGGGGGSGGGGSYVLTQPPSVSVAPGQTARITCGGNNLESKIVSWYQQKPGQAPVLVIFYDTDRPSGIPERFSGSNSGNTATLTISRVEAGDEADYYCQVWDSNSDHVVFGGGTKLTVLGSTSGSGKPGSGEGSTKGEVQLVESGGGVVQPGGSLRLSCAASGFTFDDYTMHWV

SEQ ID NO: 37 - protein, 176 aa, Artificial Sequence
  Anti-PD-L1-OX40 Ab-V11
LSLGGGGGSGGGGSYVLTQPPSVSVTPGETARIACGGNNLESKIVSWYQQKPGQAPVLVIFYDTDRPSGISERFSGSNSGNTATLTISRVEAGDEADYYCQVWDSNSDHVIFGGGTKLTVLGSTSGSGKPGSGEGSTKGEVQLVESGGVVVQPGGSLRLSCAASGFTFDDYTMHWV

SEQ ID NO: 38 - protein, 176 aa, Artificial Sequence
  Anti-PD-L1-OX40 Ab-V12
LSLGGGGGSGGGGSYVLTQPPSVSVTPGQTARIACGGNNLESKIVSWYQQKPGQAPVLVIFYDTDRPSGISERFSGSNSGNTATLTISRVEAGDEADYYCQVWDSNSDHVIFGGGTKLTVLGSTSGSGKPGSGEGSTKGEVQLVESGGVVVQPGGSLRLSCAASGFTFDDYTMHWV

SEQ ID NO: 39 - protein, 15 aa, Artificial Sequence
  linker
GGGGSGGGGSGGGGS

SEQ ID NO: 40 - protein, 19 aa, Artificial Sequence
  linker
SSGGGGSGGGGGGSSRSSL

SEQ ID NO: 41 - protein, 20 aa, Artificial Sequence
  linker
GGKGSGGKGTGGKGSGGKGS

SEQ ID NO: 42 - protein, 13 aa, Artificial Sequence
  linker
GSASAPTLFPLVS

SEQ ID NO: 43 - protein, 18 aa, Artificial Sequence
  linker
GSTSGSGKPGSGEGSTKG